European Patent Application EP 4 807 016 A1, published September 16, 2026. Title: REPORTER PROBE FOR NUCLEIC ACID DETECTION. Applicant: UNIVERSITÄTSKLINIKUM HAMBURG-EPPENDORF (UKE). Application EP. The sequence listing filed with the application follows.

SEQUENCE LISTING (36 sequences)

SEQ ID NO: 1 - DNA, 21 bp, synthetic construct
  source 1..21: mol_type = other DNA
ctgtggctaaagtcctctatg

SEQ ID NO: 2 - DNA, 22 bp, synthetic construct
  source 1..22: mol_type = other DNA
caacaacccaatctttaggaaa

SEQ ID NO: 3 - DNA, 20 bp, synthetic construct
  source 1..20: mol_type = other DNA
  modified_base 1: mod_base = OTHER; mod_base = OTHER; note = FAM
  misc_feature 9^10: note = ZEN
  modified_base 20: mod_base = OTHER; mod_base = OTHER; note = IBFQ
cgtctcccgtttggtttccg

SEQ ID NO: 4 - DNA, 35 bp, synthetic construct
  source 1..35: mol_type = other DNA
  modified_base 35: mod_base = OTHER; mod_base = OTHER; note = C3 (C3H3O4P) spacer
ggtccttcatcgctccgtctcccgtttggtttccg

SEQ ID NO: 5 - DNA, 42 bp, synthetic construct
  source 1..42: mol_type = other DNA
  modified_base 1: mod_base = OTHER; note = BHQ2
  modified_base 18: mod_base = OTHER; note = FAM-dT
  modified_base 42: mod_base = OTHER; note = C3 (C3H3O4P) spacer
ttttttttttttttttctctcttgacggagcgatgaaggacc

SEQ ID NO: 6 - DNA, 17 bp, synthetic construct
  source 1..17: mol_type = other DNA
aacacacctggcgacct

SEQ ID NO: 7 - DNA, 20 bp, synthetic construct
  source 1..20: mol_type = other DNA
caatctttaggaaaacccgc

SEQ ID NO: 8 - DNA, 30 bp, synthetic construct
  source 1..30: mol_type = other DNA
gtcgcgtctcccgtttggttttatgactct

SEQ ID NO: 9 - DNA, 63 bp, synthetic construct
  source 1..63: mol_type = other DNA
  modified_base 1: mod_base = OTHER; note = BHQ2
  modified_base 20: mod_base = OTHER; note = TexasRed-dT
  modified_base 63: mod_base = OTHER; note = C3 (C3H3O4P) spacer
aaacagcccgcggtcgttttccttttagagtcattcgatcagccacctctcaatggtgtgggt

SEQ ID NO: 10 - DNA, 38 bp, synthetic construct
  source 1..38: mol_type = other DNA
ttaggaaaacccgctcgtatttgcgcactgacgtccac

SEQ ID NO: 11 - DNA, 20 bp, synthetic construct
  source 1..20: mol_type = other DNA
cgtactgtggctaaagtcct

SEQ ID NO: 12 - DNA, 37 bp, synthetic construct
  source 1..37: mol_type = other DNA
cctgcgccaacgggtttgtaatctctctcctgggctt

SEQ ID NO: 13 - DNA, 18 bp, synthetic construct
  source 1..18: mol_type = other DNA
gccgttgtatacaccgct

SEQ ID NO: 14 - DNA, 18 bp, synthetic construct
  source 1..18: mol_type = other DNA
ccggaacgacattggttt

SEQ ID NO: 15 - DNA, 30 bp, synthetic construct; identical to SEQ ID NO: 8
  source 1..30: mol_type = other DNA

SEQ ID NO: 16 - DNA, 63 bp, synthetic construct; identical to SEQ ID NO: 9
  source 1..63: mol_type = other DNA
  modified_base 1: mod_base = OTHER; note = BHQ2
  modified_base 20: mod_base = OTHER; note = TexasRed-dT
  modified_base 63: mod_base = OTHER; note = C3 (C3H3O4P) spacer

SEQ ID NO: 17 - DNA, 17 bp, synthetic construct
  source 1..17: mol_type = other DNA
  modified_base 16: mod_base = um
agggcgtagttgtgctc

SEQ ID NO: 18 - DNA, 20 bp, synthetic construct
  source 1..20: mol_type = other DNA
  modified_base 19: mod_base = gm
gtgttcatccttaaccacgc

SEQ ID NO: 19 - DNA, 20 bp, synthetic construct
  source 1..20: mol_type = other DNA
  modified_base 19: mod_base = um
gccacaccagtgacaatatc

SEQ ID NO: 20 - DNA, 17 bp, synthetic construct
  source 1..17: mol_type = other DNA
  modified_base 15: mod_base = cm
gtgctcagtgtcggcat

SEQ ID NO: 21 - DNA, 22 bp, synthetic construct
  source 1..22: mol_type = other DNA
ccrtccaatggtctcattgtcc

SEQ ID NO: 22 - DNA, 22 bp, synthetic construct
  source 1..22: mol_type = other DNA
tcgtctaatggrcttatcgtcc

SEQ ID NO: 23 - DNA, 17 bp, synthetic construct
  source 1..17: mol_type = other DNA
gccgacgcggtcgtcat

SEQ ID NO: 24 - DNA, 19 bp, synthetic construct
  source 1..19: mol_type = other DNA
ccaccgactcgatcgtcat

SEQ ID NO: 25 - DNA, 40 bp, synthetic construct
  source 1..40: mol_type = other DNA
gaataagcagcaaggatttaccaataatctttttcctacg

SEQ ID NO: 26 - DNA, 59 bp, synthetic construct
  source 1..59: mol_type = other DNA
  modified_base 1: mod_base = OTHER; note = BHQ2
  modified_base 21: mod_base = OTHER; note = JOE-dT
  modified_base 59: mod_base = OTHER; note = C3 (C3H3O4P) spacer
cgttccgtcttttttttttcttcttcgtaggaataacgggcgaaccaagcatttttacc

SEQ ID NO: 27 - DNA, 27 bp, synthetic construct
  source 1..27: mol_type = other DNA
gcgacttggccttgctgtaaacctgag

SEQ ID NO: 28 - DNA, 59 bp, synthetic construct
  source 1..59: mol_type = other DNA
  modified_base 1: mod_base = OTHER; note = BHQ2
  modified_base 21: mod_base = OTHER; note = JOE-dT
  modified_base 59: mod_base = OTHER; note = C3 (C3H3O4P) spacer
gccgtgctcgtcgtcctccttctctctcaggttacttgatcaggcagccaccaaaagcg

SEQ ID NO: 29 - DNA, 29 bp, synthetic construct
  source 1..29: mol_type = other DNA
  modified_base 1: mod_base = OTHER; note = SUN
  modified_base 9^10: mod_base = OTHER; note = ZEN
  modified_base 29: mod_base = OTHER; note = IBFQ
atgagttgcttttgattgatacagcktgg

SEQ ID NO: 30 - DNA, 18 bp, synthetic construct
  source 1..18: mol_type = other DNA
ctggaatgccgcctacaa

SEQ ID NO: 31 - DNA, 19 bp, synthetic construct
  source 1..19: mol_type = other DNA
gttgccctgtccgtctatc

SEQ ID NO: 32 - DNA, 32 bp, synthetic construct
  source 1..32: mol_type = other DNA
cggtaaataccacccccacggcttatgctcta

SEQ ID NO: 33 - DNA, 57 bp, synthetic construct
  source 1..57: mol_type = other DNA
  modified_base 1: mod_base = OTHER; note = BHQ2
  modified_base 20: mod_base = OTHER; note = JOE-dT
  modified_base 39: mod_base = OTHER; note = LNA cytosine
  modified_base 57: mod_base = OTHER; note = C3 (C3H3O4P) spacer
aaagtgccggtcttttttcttttcttagagcatatattccgcagtttacgvcaccat

SEQ ID NO: 34 - DNA, 58 bp, synthetic construct
  source 1..58: mol_type = other DNA
  modified_base 1: mod_base = OTHER; note = BHQ2
  modified_base 20: mod_base = OTHER; note = JOE-dT
  modified_base 39: mod_base = OTHER; note = LNA thymine
  modified_base 58: mod_base = OTHER; note = C3 (C3H3O4P) spacer
aaactcgccgcggtcctcctttttctagagcatatatttcgcagtttacgvcaccatc

SEQ ID NO: 35 - DNA, 63 bp, Klebsiella pneumoniae
  source 1..63: mol_type = other DNA
gtccacctcgacccacaccattgagaggtggctgatcggaaaccaaacgggagacgcgacact

SEQ ID NO: 36 - DNA, 63 bp, Klebsiella pneumoniae
  source 1..63: mol_type = other DNA
agtgtcgcgtctcccgtttggtttccgatcagccacctctcaatggtgtgggtcgaggtggac